European Patent Specification EP 3 915 397 B1, published November 20, 2024. Title: USE OF A SWEET PROTEIN FOR EHANCING THE SWEET TASTE AND/OR SWEET QUALITY. Applicant: BRAIN AG. The sequence listing filed with the application follows.

SEQUENCE LISTING (4 sequences)

SEQ ID NO: 1 - protein, 53 aa, Unknown
  Artificial Sequence
DKCKKVYENYPVSKCQLANQCNYDCKLDKHARSGECFYDEKRNLQCICDYCEY

SEQ ID NO: 2 - DNA, 162 bp, Unknown
  Artificial Sequence
gataagtgtaaaaaggtttacgaaaactatccagtgtctaaatgccaactggcaaatcagtgtaattacgattgtaaattggataagcatgctagatccggtgaatgtttctacgacgagaagcgtaacttacaatgtatctgcgactattgtgagtattag

SEQ ID NO: 3 - DNA, 417 bp, Unknown
  Artificial Sequence
atgagattcccatctattttcaccgctgtcttgttcgctgcctcctctgcattggctgcccctgttaacactaccactgaagacgagactgctcaaattccagctgaagcagttatcggttactctgaccttgagggtgatttcgacgtcgctgttttgcctttctctaactccactaacaacggtttgttgttcattaacaccactatcgcttccattgctgctaaggaagagggtgtctctctcgagaaaagagataagtgtaaaaaggtttacgaaaactatccagtgtctaaatgccaactggcaaatcagtgtaattacgattgtaaattggataagcatgctagatccggtgaatgtttctacgacgagaagcgtaacttacaatgtatctgcgactattgtgagtattag

SEQ ID NO: 4 - DNA, 1634 bp, Unknown
  Artificial Sequence
aacatccaaagacgaaaggttgaatgaaacctttttgccatccgacatccacaggtccattctcacacataagtgccaaacgcaacaggaggggatacactagcagcagaccgttgcaaacgcaggacctccactcctcttctcctcaacacccacttttgccatcgaaaaaccagcccagttattgggcttgattggagctcgctcattccaattccttctattaggctactaacaccatgactttattagcctgtctatcctggcccccctggcgaggttcatgtttgtttatttccgaatgcaacaagctccgcattacacccgaacatcactccagatgagggctttctgagtgtggggtcaaatagtttcatgttccccaaatggcccaaaactgacagtttaaacgctgtcttggaacctaatatgacaaaagcgtgatctcatccaagatgaactaagtttggttcgttgaaatgctaacggccagttggtcaaaaagaaacttccaaaagtcggcataccgtttgtcttgtttggtattgattgacgaatgctcaaaaataatctcattaatgcttagcgcagtctctctatcgcttctgaaccccggtgcacctgtgccgaaacgcaaatggggaaacacccgctttttggatgattatgcattgtctccacattgtatgcttccaagattctggtgggaatactgctgatagcctaacgttcatgatcaaaatttaactgttctaacccctacttgacagcaatatataaacagaaggaagctgccctgtcttaaacctttttttttatcatcattattagcttactttcataattgcgactggttccaattgacaagcttttgattttaacgacttttaacgacaacttgagaagatcaaaaaacaactaattattgaaagaattccgaaacgatgagattcccatctattttcaccgctgtcttgttcgctgcctcctctgcattggctgcccctgttaacactaccactgaagacgagactgctcaaattccagctgaagcagttatcggttactctgaccttgagggtgatttcgacgtcgctgttttgcctttctctaactccactaacaacggtttgttgttcattaacaccactatcgcttccattgctgctaaggaagagggtgtctctctcgagaaaagagataagtgtaaaaaggtttacgaaaactatccagtgtctaaatgccaactggcaaatcagtgtaattacgattgtaaattggataagcatgctagatccggtgaatgtttctacgacgagaagcgtaacttacaatgtatctgcgactattgtgagtattagtaagcggccgctcaagaggatgtcagaatgccatttgcctgagagatgcaggcttcatttttgatacttttttatttgtaacctatatagtataggattttttttgtcattttgtttcttctcgtacgagcttgctcctgatcagcctatctcgcagcagatgaatatcttgtggtaggggtttgggaaaatcattcgagtttgatgtttttcttggtatttcccactcctcttcagagtacagaagattaagtgagaccttcgtttgtgcgg